European Patent Application EP 4 159 863 A1, published April 5, 2023. Title: Codon-optimized nucleic acid that encodes SMN1 protein, and use thereof. Applicant: LLC "ANABION". Application PCT/RU2021/000238. The sequence listing filed with the application follows.

SEQUENCE LISTING (13 sequences)

SEQ ID NO: 1 - protein, 294 aa, Natural sequence
  The amino acid sequence of the SMN1 protein
MAMSSGGSGGGVPEQEDSVLFRRGTGQSDDSDIWDDTALIKAYDKAVASFKHALKNGDICETSGKPKTTPKRKPAKKNKSQKKNTAASLQQWKVGDKCSAIWSEDGCIYPATIASIDFKRETCVVVYTGYGNREEQNLSDLLSPICEVANNIEQNAQENENESQVSTDESENSRSPGNKSDNIKPKSAPWNSFLPPPPPMPGPRLGPGKPGLKFNGPPPPPPPPPPHLLSCWLPPFPSGPPIIPPPPPICPDSLDDADALGSMLISWYMSGYHTGYYMGFRQNQKEGRCSHSLN

SEQ ID NO: 2 - DNA, 882 bp, Artificial sequence
  Codon-an optimized nucleic acid sequence that encodes the SMN1 protein (SMN1 GeneBeam)
atggccatgagcagcggcggcagcggcggcggcgtgcctgagcaagaggacagcgtgctgttcagaagaggcaccggccagagcgacgacagcgacatctgggacgacaccgccctgatcaaggcctacgacaaggccgtggccagcttcaagcacgccctgaagaacggcgacatctgcgagaccagcggcaagcccaagaccacccccaagagaaagcccgccaagaagaacaagagccagaagaagaacaccgccgccagcctgcagcagtggaaggtgggcgacaagtgcagcgccatctggagcgaggacggctgcatctaccccgccaccatcgccagcatcgacttcaagagagagacctgcgtggtggtgtacaccggctacggcaacagagaggagcagaacctgagcgacctgctgagccccatctgcgaggtggccaacaacatcgagcagaacgcccaagagaacgagaacgagagccaagtgagcaccgacgagagcgagaacagcagaagccccggcaacaagagcgacaacatcaagcccaagagcgccccctggaacagcttcctgccccctcccccccctatgcccggccctagactgggccctggcaagcctggcctgaagttcaacggcccccccccccctcctcctcctcctcctcctcacctgctgagctgctggctgccccccttccccagcggccctcctatcatccctcctcccccccccatctgccccgacagcctggacgacgccgacgccctgggcagcatgctgatcagctggtacatgagcggctaccacaccggctactacatgggcttcagacagaaccagaaggagggccggtgcagccacagcctgaac

SEQ ID NO: 3 - DNA, 885 bp, Natural sequence
  The nucleic acid sequence of the wild-type SMN1 gene (SMN1-WT, SMN1-Wild type)
atggcgatgagcagcggcggcagtggtggcggcgtcccggagcaggaggattccgtgctgttccggcgcggcacaggccagagcgatgattctgacatttgggatgatacagcactgataaaagcatatgataaagctgtggcttcatttaagcatgctctaaagaatggtgacatttgtgaaacttcgggtaaaccaaaaaccacacctaaaagaaaacctgctaagaagaataaaagccaaaagaagaatactgcagcttccttacaacagtggaaagttggggacaaatgttctgccatttggtcagaagacggttgcatttacccagctaccattgcttcaattgattttaagagagaaacctgtgttgtggtttacactggatatggaaatagagaggagcaaaatctgtccgatctactttccccaatctgtgaagtagctaataatatagaacaaaatgctcaagagaatgaaaatgaaagccaagtttcaacagatgaaagtgagaactccaggtctcctggaaataaatcagataacatcaagcccaaatctgctccatggaactcttttctccctccaccaccccccatgccagggccaagactgggaccaggaaagccaggtctaaaattcaatggcccaccaccgccaccgccaccaccaccaccccacttactatcatgctggctgcctccatttccttctggaccaccaataattcccccaccacctcccatatgtccagattctcttgatgatgctgatgctttgggaagtatgttaatttcatggtacatgagtggctatcatactggctattatatgggtttcagacaaaatcaaaaagaaggaaggtgctcacattccttaaattaa

SEQ ID NO: 4 - DNA, 2924 bp, Artificial sequence
  The nucleic acid sequence of the expression cassette (complete)
cctgcaggcagctgcgcgctcgctcgctcactgaggccgcccgggcgtcgggcgacctttggtcgcccggcctcagtgagcgagcgagcgcgcagagagggagtggccaactccatcactaggggttcctgcggccgcacgcgtctagttattaatagtaatcaattacggggtcattagttcatagcccatatatggagttccgcgttacataacttacggtaaatggcccgcctggctgaccgcccaacgacccccgcccattgacgtcaataatgacgtatgttcccatagtaacgccaatagggactttccattgacgtcaatgggtggagtatttacggtaaactgcccacttggcagtacatcaagtgtatcatatgccaagtacgccccctattgacgtcaatgacggtaaatggcccgcctggcattatgcccagtacatgaccttatgggactttcctacttggcagtacatctacgtattagtcatcgctattaccatggtgatgcggttttggcagtacatcaatgggcgtggatagcggtttgactcacggggatttccaagtctccaccccattgacgtcaatgggagtttgttttggcaccaaaatcaacgggactttccaaaatgtcgtaacaactccgccccattgacgcaaatgggcggtaggcgtgtacggtgggaggtctatataagcagagctcgtttagtgaaccgtcagatcgcctggagacgccatccacgctgttttgacctccatagaagacaccgggaccgatccagcctccgcggattcgaatcccggccgggaacggtgcattggaacgcggattccccgtgccaagagtgacgtaagtaccgcctatagagtctataggcccacaaaaaatgctttcttcttttaatatacttttttgtttatcttatttctaatactttccctaatctctttctttcagggcaataatgatacaatgtatcatgcctctttgcaccattctaaagaataacagtgataatttctgggttaaggcaatagcaatatttctgcatataaatatttctgcatataaattgtaactgatgtaagaggtttcatattgctaatagcagctacaatccagctaccattctgcttttattttatggttgggataaggctggattattctgagtccaagctaggcccttttgctaatcatgttcatacctcttatcttcctcccacagctcctgggcaacgtgctggtctgtgtgctggcccatcactttggcaaagaattgggattcgaacatcgattgtaattcatgagccaccatggccatgagcagcggcggcagcggcggcggcgtgcctgagcaagaggacagcgtgctgttcagaagaggcaccggccagagcgacgacagcgacatctgggacgacaccgccctgatcaaggcctacgacaaggccgtggccagcttcaagcacgccctgaagaacggcgacatctgcgagaccagcggcaagcccaagaccacccccaagagaaagcccgccaagaagaacaagagccagaagaagaacaccgccgccagcctgcagcagtggaaggtgggcgacaagtgcagcgccatctggagcgaggacggctgcatctaccccgccaccatcgccagcatcgacttcaagagagagacctgcgtggtggtgtacaccggctacggcaacagagaggagcagaacctgagcgacctgctgagccccatctgcgaggtggccaacaacatcgagcagaacgcccaagagaacgagaacgagagccaagtgagcaccgacgagagcgagaacagcagaagccccggcaacaagagcgacaacatcaagcccaagagcgccccctggaacagcttcctgccccctcccccccctatgcccggccctagactgggccctggcaagcctggcctgaagttcaacggcccccccccccctcctcctcctcctcctcctcacctgctgagctgctggctgccccccttccccagcggccctcctatcatccctcctcccccccccatctgccccgacagcctggacgacgccgacgccctgggcagcatgctgatcagctggtacatgagcggctaccacaccggctactacatgggcttcagacagaaccagaaggagggccggtgcagccacagcctgaactgatctagagtcgacctgcagaagcttgcctcgagcagcgctgctcgagagatctacgggtggcatccctgtgacccctccccagtgcctctcctggccctggaagttgccactccagtgcccaccagccttgtcctaataaaattaagttgcatcattttgtctgactaggtgtccttctataatattatggggtggaggggggtggtatggagcaaggggcaagttgggaagacaacctgtagggcctgcggggtctattgggaaccaagctggagtgcagtggcacaatcttggctcactgcaatctccgcctcctgggttcaagcgattctcctgcctcagcctcccgagttgttgggattccaggcatgcatgaccaggctcagctaatttttgtttttttggtagagacggggtttcaccatattggccaggctggtctccaactcctaatctcaggtgatctacccaccttggcctcccaaattgctgggattacaggcgtgaaccactgctcccttccctgtccttctgattttgtaggtaaccacgtgcggaccgagcggccgcaggaacccctagtgatggagttggccactccctctctgcgcgctcgctcgctcactgaggccgggcgaccaaaggtcgcccgacgcccgggctttgcccgggcggcctcagtgagcgagcgagcgcgcagctgcctgcagg

SEQ ID NO: 5 - protein, 736 aa, Natural sequence
  The amino acid sequence of the VP1 AAV9 protein
MAADGYLPDWLEDNLSEGIREWWALKPGAPQPKANQQHQDNARGLVLPGYKYLGPGNGLDKGEPVNAADAAALEHDKAYDQQLKAGDNPYLKYNHADAEFQERLKEDTSFGGNLGRAVFQAKKRLLEPLGLVEEAAKTAPGKKRPVEQSPQEPDSSAGIGKSGAQPAKKRLNFGQTGDTESVPDPQPIGEPPAAPSGVGSLTMASGGGAPVADNNEGADGVGSSSGNWHCDSQWLGDRVITTSTRTWALPTYNNHLYKQISNSTSGGSSNDNAYFGYSTPWGYFDFNRFHCHFSPRDWQRLINNNWGFRPKRLNFKLFNIQVKEVTDNNGVKTIANNLTSTVQVFTDSDYQLPYVLGSAHEGCLPPFPADVFMIPQYGYLTLNDGSQAVGRSSFYCLEYFPSQMLRTGNNFQFSYEFENVPFHSSYAHSQSLDRLMNPLIDQYLYYLSKTINGSGQNQQTLKFSVAGPSNMAVQGRNYIPGPSYRQQRVSTTVTQNNNSEFAWPGASSWALNGRNSLMNPGPAMASHKEGEDRFFPLSGSLIFGKQGTGRDNVDADKVMITNEEEIKTTNPVATESYGQVATNHQSAQAQAQTGWVQNQGILPGMVWQDRDVYLQGPIWAKIPHTDGNFHPSPLMGGFGMKHPPPQILIKNTPVPADPPTAFNKDKLNSFITQYSTGQVSVEIEWELQKENSKRWNPEIQYTSNYYKSNNVEFAVNTEGVYSEPRPIGTRYLTRNL

SEQ ID NO: 6 - protein, 599 aa, Natural sequence
  The amino acid sequence of the VP2 AAV9 protein
TAPGKKRPVEQSPQEPDSSAGIGKSGAQPAKKRLNFGQTGDTESVPDPQPIGEPPAAPSGVGSLTMASGGGAPVADNNEGADGVGSSSGNWHCDSQWLGDRVITTSTRTWALPTYNNHLYKQISNSTSGGSSNDNAYFGYSTPWGYFDFNRFHCHFSPRDWQRLINNNWGFRPKRLNFKLFNIQVKEVTDNNGVKTIANNLTSTVQVFTDSDYQLPYVLGSAHEGCLPPFPADVFMIPQYGYLTLNDGSQAVGRSSFYCLEYFPSQMLRTGNNFQFSYEFENVPFHSSYAHSQSLDRLMNPLIDQYLYYLSKTINGSGQNQQTLKFSVAGPSNMAVQGRNYIPGPSYRQQRVSTTVTQNNNSEFAWPGASSWALNGRNSLMNPGPAMASHKEGEDRFFPLSGSLIFGKQGTGRDNVDADKVMITNEEEIKTTNPVATESYGQVATNHQSAQAQAQTGWVQNQGILPGMVWQDRDVYLQGPIWAKIPHTDGNFHPSPLMGGFGMKHPPPQILIKNTPVPADPPTAFNKDKLNSFITQYSTGQVSVEIEWELQKENSKRWNPEIQYTSNYYKSNNVEFAVNTEGVYSEPRPIGTRYLTRNL

SEQ ID NO: 7 - protein, 534 aa, Natural sequence
  The amino acid sequence of the VP3 AAV9 protein
MASGGGAPVADNNEGADGVGSSSGNWHCDSQWLGDRVITTSTRTWALPTYNNHLYKQISNSTSGGSSNDNAYFGYSTPWGYFDFNRFHCHFSPRDWQRLINNNWGFRPKRLNFKLFNIQVKEVTDNNGVKTIANNLTSTVQVFTDSDYQLPYVLGSAHEGCLPPFPADVFMIPQYGYLTLNDGSQAVGRSSFYCLEYFPSQMLRTGNNFQFSYEFENVPFHSSYAHSQSLDRLMNPLIDQYLYYLSKTINGSGQNQQTLKFSVAGPSNMAVQGRNYIPGPSYRQQRVSTTVTQNNNSEFAWPGASSWALNGRNSLMNPGPAMASHKEGEDRFFPLSGSLIFGKQGTGRDNVDADKVMITNEEEIKTTNPVATESYGQVATNHQSAQAQAQTGWVQNQGILPGMVWQDRDVYLQGPIWAKIPHTDGNFHPSPLMGGFGMKHPPPQILIKNTPVPADPPTAFNKDKLNSFITQYSTGQVSVEIEWELQKENSKRWNPEIQYTSNYYKSNNVEFAVNTEGVYSEPRPIGTRYLTRNL

SEQ ID NO: 8 - DNA, 130 bp, Natural sequence
  Left (first) ITR (inverted end repeats)
cctgcaggcagctgcgcgctcgctcgctcactgaggccgcccgggcgtcgggcgacctttggtcgcccggcctcagtgagcgagcgagcgcgcagagagggagtggccaactccatcactaggggttcct

SEQ ID NO: 9 - DNA, 304 bp, Natural sequence
  CMV (Cytomegalovirus) Enhancer
cgttacataacttacggtaaatggcccgcctggctgaccgcccaacgacccccgcccattgacgtcaataatgacgtatgttcccatagtaacgccaatagggactttccattgacgtcaatgggtggagtatttacggtaaactgcccacttggcagtacatcaagtgtatcatatgccaagtacgccccctattgacgtcaatgacggtaaatggcccgcctggcattatgcccagtacatgaccttatgggactttcctacttggcagtacatctacgtattagtcatcgctattaccatg

SEQ ID NO: 10 - DNA, 204 bp, Natural sequence
  CMV (Cytomegalovirus) promoter
gtgatgcggttttggcagtacatcaatgggcgtggatagcggtttgactcacggggatttccaagtctccaccccattgacgtcaatgggagtttgttttggcaccaaaatcaacgggactttccaaaatgtcgtaacaactccgccccattgacgcaaatgggcggtaggcgtgtacggtgggaggtctatataagcagagct

SEQ ID NO: 11 - DNA, 493 bp, Natural sequence
  Intron of the hBG1 gene (hemoglobin gamma-1 subunit)
cgaatcccggccgggaacggtgcattggaacgcggattccccgtgccaagagtgacgtaagtaccgcctatagagtctataggcccacaaaaaatgctttcttcttttaatatacttttttgtttatcttatttctaatactttccctaatctctttctttcagggcaataatgatacaatgtatcatgcctctttgcaccattctaaagaataacagtgataatttctgggttaaggcaatagcaatatttctgcatataaatatttctgcatataaattgtaactgatgtaagaggtttcatattgctaatagcagctacaatccagctaccattctgcttttattttatggttgggataaggctggattattctgagtccaagctaggcccttttgctaatcatgttcatacctcttatcttcctcccacagctcctgggcaacgtgctggtctgtgtgctggcccatcactttggcaaagaattgggat

SEQ ID NO: 12 - DNA, 479 bp, Natural sequence
  hGH1 polyadenylation signal (polyadenylation signal(poly (A)) of Human Growth Hormone)
acgggtggcatccctgtgacccctccccagtgcctctcctggccctggaagttgccactccagtgcccaccagccttgtcctaataaaattaagttgcatcattttgtctgactaggtgtccttctataatattatggggtggaggggggtggtatggagcaaggggcaagttgggaagacaacctgtagggcctgcggggtctattgggaaccaagctggagtgcagtggcacaatcttggctcactgcaatctccgcctcctgggttcaagcgattctcctgcctcagcctcccgagttgttgggattccaggcatgcatgaccaggctcagctaatttttgtttttttggtagagacggggtttcaccatattggccaggctggtctccaactcctaatctcaggtgatctacccaccttggcctcccaaattgctgggattacaggcgtgaaccactgctcccttccctgtcctt

SEQ ID NO: 13 - DNA, 141 bp, Natural sequence
  Right (second) ITR
aggaacccctagtgatggagttggccactccctctctgcgcgctcgctcgctcactgaggccgggcgaccaaaggtcgcccgacgcccgggctttgcccgggcggcctcagtgagcgagcgagcgcgcagctgcctgcagg